European Patent Specification EP 4 058 448 B1, published May 29, 2024. Title: SUBSTITUTED HYDANTOINAMIDES AND THEIR USE / ASSAY FOR CHARACTERIZATION OF ADAMTS-7 AND/OR ADAMTS-12 MODULATORS. Applicant: Bayer AG BROAD Institute. The sequence listing filed with the application follows.

SEQUENCE LISTING (33 sequences)

SEQ ID NO: 1 - protein, 562 aa, Artificial Sequence
  rPro-hCD (Rat 1-217/Human 237-537)-TEV-2Strep-6His
  ADAMTS7 rat prodomain (wild-type) (1)..(217)
  ADAMTS7 human catalytic domain (218)..(518)
  TEV cleavage site, 2xStrep tag, and a His tag (519)..(562)
MHRGLNLLLILCALAPHVLGPASGLPTEGRAGLDIVHPVRVDAGGSFLSYELWPRVLRKRDVSAAQASSAFYQLQYQGRELLFNLTTNPYLLAPGFVSEIRRRSNLSNVHIQTSVPTCHLLGDVQDPELEGGFAAISACDGLRGVFQLSNEDYFIEPLDEVPAQPGHAQPHMVYKHKRSGQQDDSRTSGTCGVQGSPELKHQREHWEQRQQKRRQQRSVSKEKWVETLVVADAKMVEYHGQPQVESYVLTIMNMVAGLFHDPSIGNPIHITIVRLVLLEDEEEDLKITHHADNTLKSFCKWQKSINMKGDAHPLHHDTAILLTRKDLCAAMNRPCETLGLSHVAGMCQPHRSCSINEDTGLPLAFTVAHELGHSFGIQHDGSGNDCEPVGKRPFIMSPQLLYDAAPLTWSRCSRQYITRFLDRGWGLCLDDPPAKDIIDFPSVPPGVLYDVSHQCRLQYGAYSAFCEDMDNVCHTLWCSVGTTCHSKLDAAVDGTRCGENKWCLSGECVPVGFRPEAVGSENLYFQSGWSHPQFEKGGGSGGGSGGGSWSHPQFEKHHHHHH

SEQ ID NO: 2 - protein, 562 aa, Artificial Sequence
  rPro-hCD-FM2 (Rat 1-217/Human 237-537 FM2 (Q216K))-TEV-2Strep-6His
  ADAMTS7 rat prodomain (furin mutant Q216K) (1)..(217)
  ADAMTS7 human catalytic domain (218)..(518)
  TEV cleavage site, 2xStrep tag, and a His tag (519)..(562)
MHRGLNLLLILCALAPHVLGPASGLPTEGRAGLDIVHPVRVDAGGSFLSYELWPRVLRKRDVSAAQASSAFYQLQYQGRELLFNLTTNPYLLAPGFVSEIRRRSNLSNVHIQTSVPTCHLLGDVQDPELEGGFAAISACDGLRGVFQLSNEDYFIEPLDEVPAQPGHAQPHMVYKHKRSGQQDDSRTSGTCGVQGSPELKHQREHWEQRQQKRRQKRSVSKEKWVETLVVADAKMVEYHGQPQVESYVLTIMNMVAGLFHDPSIGNPIHITIVRLVLLEDEEEDLKITHHADNTLKSFCKWQKSINMKGDAHPLHHDTAILLTRKDLCAAMNRPCETLGLSHVAGMCQPHRSCSINEDTGLPLAFTVAHELGHSFGIQHDGSGNDCEPVGKRPFIMSPQLLYDAAPLTWSRCSRQYITRFLDRGWGLCLDDPPAKDIIDFPSVPPGVLYDVSHQCRLQYGAYSAFCEDMDNVCHTLWCSVGTTCHSKLDAAVDGTRCGENKWCLSGECVPVGFRPEAVGSENLYFQSGWSHPQFEKGGGSGGGSGGGSWSHPQFEKHHHHHH

SEQ ID NO: 3 - protein, 573 aa, Artificial Sequence
  rADAMTS7 (Rat 1-575)-Flag
MPCAQGNWMAKLSMVAQLLNFGAFCHGRQAQPWPVRFPDPKQEHFIKSLPEYHIVSPVQVDASGHFLSYGLHHPVTGSRKKRAAGGSGDQVYYRISHEEKNLFFNLTVNWEFLSNGYVVERRYGNLSHVKMAASSGQPCHLRGTVLQQGPTIRMGTAALSACQGLTGFFHLPHGDFFIEPVKKHPLTEEGYQPHVIYRRQSYRVPETKEPTCGLKDSLDNSVKQELQREKWERKNWPSRSLSRRSISKERWVETLVVADTKMIEYHGSENVESYILTIMNMVTGLFHNPSIGNAIHIVVVRLILLEEEEQGLKIVHHAEKTLSSFCKWQKSINPKSDLNPVHHDVAVLLTRKDICAGFNRPCETLGLSHLSGMCQPHRSCNINEDSGLPLAFTIAHELGHSFGIQHDGKENDCEPVGRHPYIMSRQLQYDPTPLTWSKCSEEYITRFLDRGWGFCLDDIPKKKGLKSKVIAPGVIYDVHHQCQLQYGPNATFCQEVENVCQTLWCSVKGFCRSKLDAAADGTQCGEKKWCMAGKCITVGKKPESIPGGGGSDYKDHDGDYKDHDIDYKDDDDK

SEQ ID NO: 4 - protein, 16 aa, Artificial Sequence
  Test substrate for ADAMTS7/12: (HiLyteFluor-488 )-DELSSMVLELRGLRT-K(QXL520)-NH2
DELSSMVLELRGLRTK

SEQ ID NO: 5 - protein, 16 aa, Artificial Sequence
  Test Substrate for ADAMTS7/12: (HiLyteFluor-488)-SSMVLELRGLRTIVT-K(QXL520)-NH2
SSMVLELRGLRTIVTK

SEQ ID NO: 6 - protein, 16 aa, Artificial Sequence
  Test Substrate for ADAMTS7/12: (HiLyteFluor-488)-KVTEENKELANELRR-K(QXL520)-NH2
KVTEENKELANELRRK

SEQ ID NO: 7 - protein, 16 aa, Artificial Sequence
  Test Substrate for ADAMTS7/12: (HiLyteFluor-488)-EENKELANELRRPPL-K(QXL520)-NH2
EENKELANELRRPPLK

SEQ ID NO: 8 - protein, 13 aa, Artificial Sequence
  Test Substrate for ADAMTS7/12: (HiLyteFluor-488)-SSMVLELRGLRT-K(QXL520)-NH2
SSMVLELRGLRTK

SEQ ID NO: 9 - protein, 12 aa, Artificial Sequence
  Test Substrate for ADAMTS7/12: (Donor) GMQQSVRTGLPS (K-Quencher)
GMQQSVRTGLPS

SEQ ID NO: 10 - protein, 14 aa, Artificial Sequence
  Test Substrate for ADAMTS7/12: (Donor) SPGFRCEACPPGYS (K-Quencher)
SPGFRCEACPPGYS

SEQ ID NO: 11 - protein, 16 aa, Artificial Sequence
  Substrate for ADAMTS7 and for ADAMTS12: (HiLyteFluor-488)-DELSSMVLELRGLRT-K(QXL520)-E-NH2
DELSSMVLELRGLRTK

SEQ ID NO: 12 - protein, 16 aa, Artificial Sequence
  Test Substrate for ADAMTS7/12: (HiLyteFluor-488)-DELSSMVLELRGLRT-K(QXL520)-K-NH2
DELSSMVLELRGLRTK

SEQ ID NO: 13 - protein, 16 aa, Artificial Sequence
  Test Substrate for ADAMTS7/12: (HiLyteFluor-488)-DELSSMVLELRGLRT-K(QXL520)-OH
DELSSMVLELRGLRTK

SEQ ID NO: 14 - protein, 10 aa, Artificial Sequence
  Substrate for ADAMTS4 and for ADAMTS5: Dabcyl-EEVKAKVQPY-Glu(Edans)-NH2
EEVKAKVQPY

SEQ ID NO: 15 - protein, 573 aa, Artificial Sequence; identical to SEQ ID NO: 3
  rPro-hCD for ADAMTS12

SEQ ID NO: 16 - protein, 14 aa, Artificial Sequence
  ADAMTS Catalytic Motif Consensus Sequence
  misc_feature (3)..(4): Xaa can be any naturally occurring amino acid
  misc_feature (6)..(6): Xaa can be any naturally occurring amino acid
  misc_feature (12)..(12): Xaa can be any naturally occurring amino acid
HEXXHXBGNSBXHD

SEQ ID NO: 17 - protein, 7 aa, Artificial Sequence
  Substrate for MMP12: Mca-Pro-Leu-Gly-Leu-Glu-Glu-Ala-Dap(Dnp)-NH2
PLGLEEA

SEQ ID NO: 18 - protein, 8 aa, Artificial Sequence
  Substrate for MMP15: MCA-Lys-Pro-Leu-Gly-Leu-DPA-Ala-Arg-NH2
  X (6)..(6): DPA
KPLGLXAR

SEQ ID NO: 19 - protein, 7 aa, Artificial Sequence
  Substrate for MMP2: MCA-Pro-Leu-Gly-Leu-DPA-Ala-Arg-NH2
  X (5)..(5): DPA
PLGLXAR

SEQ ID NO: 20 - protein, 12 aa, Artificial Sequence
  Substrate for ADAM17: Mca-Pro-Leu-Ala-Gln-Ala-Val-Dap(Dnp)-Arg-Ser-Ser-Ser-Arg-NH2
  X (7)..(7): Dap(Dnp)
PLAQAVXRSSSR

SEQ ID NO: 21 - protein, 1686 aa, Artificial Sequence
  Human ADAMTS7 from Q9UKP4
MPGGPSPRSPAPLLRPLLLLLCALAPGAPGPAPGRATEGRAALDIVHPVRVDAGGSFLSYELWPRALRKRDVSVRRDAPAFYELQYRGRELRFNLTANQHLLAPGFVSETRRRGGLGRAHIRAHTPACHLLGEVQDPELEGGLAAISACDGLKGVFQLSNEDYFIEPLDSAPARPGHAQPHVVYKRQAPERLAQRGDSSAPSTCGVQVYPELESRRERWEQRQQWRRPRLRRLHQRSVSKEKWVETLVVADAKMVEYHGQPQVESYVLTIMNMVAGLFHDPSIGNPIHITIVRLVLLEDEEEDLKITHHADNTLKSFCKWQKSINMKGDAHPLHHDTAILLTRKDLCAAMNRPCETLGLSHVAGMCQPHRSCSINEDTGLPLAFTVAHELGHSFGIQHDGSGNDCEPVGKRPFIMSPQLLYDAAPLTWSRCSRQYITRFLDRGWGLCLDDPPAKDIIDFPSVPPGVLYDVSHQCRLQYGAYSAFCEDMDNVCHTLWCSVGTTCHSKLDAAVDGTRCGENKWCLSGECVPVGFRPEAVDGGWSGWSAWSICSRSCGMGVQSAERQCTQPTPKYKGRYCVGERKRFRLCNLQACPAGRPSFRHVQCSHFDAMLYKGQLHTWVPVVNDVNPCELHCRPANEYFAEKLRDAVVDGTPCYQVRASRDLCINGICKNVGCDFEIDSGAMEDRCGVCHGNGSTCHTVSGTFEEAEGLGYVDVGLIPAGAREIRIQEVAEAANFLALRSEDPEKYFLNGGWTIQWNGDYQVAGTTFTYARRGNWENLTSPGPTKEPVWIQLLFQESNPGVHYEYTIHREAGGHDEVPPPVFSWHYGPWTKCTVTCGRGVQRQNVYCLERQAGPVDEEHCDPLGRPDDQQRKCSEQPCPARWWAGEWQLCSSSCGPGGLSRRAVLCIRSVGLDEQSALEPPACEHLPRPPTETPCNRHVPCPATWAVGNWSQCSVTCGEGTQRRNVLCTNDTGVPCDEAQQPASEVTCSLPLCRWPLGTLGPEGSGSGSSSHELFNEADFIPHHLAPRPSPASSPKPGTMGNAIEEEAPELDLPGPVFVDDFYYDYNFINFHEDLSYGPSEEPDLDLAGTGDRTPPPHSHPAAPSTGSPVPATEPPAAKEEGVLGPWSPSPWPSQAGRSPPPPSEQTPGNPLINFLPEEDTPIGAPDLGLPSLSWPRVSTDGLQTPATPESQNDFPVGKDSQSQLPPPWRDRTNEVFKDDEEPKGRGAPHLPPRPSSTLPPLSPVGSTHSSPSPDVAELWTGGTVAWEPALEGGLGPVDSELWPTVGVASLLPPPIAPLPEMKVRDSSLEPGTPSFPTPGPGSWDLQTVAVWGTFLPTTLTGLGHMPEPALNPGPKGQPESLSPEVPLSSRLLSTPAWDSPANSHRVPETQPLAPSLAEAGPPADPLVVRNAGWQAGNWSECSTTCGLGAVWRPVRCSSGRDEDCAPAGRPQPARRCHLRPCATWHSGNWSKCSRSCGGGSSVRDVQCVDTRDLRPLRPFHCQPGPAKPPAHRPCGAQPCLSWYTSSWRECSEACGGGEQQRLVTCPEPGLCEEALRPNTTRPCNTHPCTQWVVGPWGQCSGPCGGGVQRRLVKCVNTQTGLPEEDSDQCGHEAWPESSRPCGTEDCEPVEPPRCERDRLSFGFCETLRLLGRCQLPTIRTQCCRSCSPPSHGAPSRGHQRVARR

SEQ ID NO: 22 - protein, 1595 aa, Artificial Sequence
  Rat ADAMTS7 from Q1EHB3
MHRGLNLLLILCALAPHVLGPASGLPTEGRAGLDIVHPVRVDAGGSFLSYELWPRVLRKRDVSAAQASSAFYQLQYQGRELLFNLTTNPYLLAPGFVSEIRRRSNLSNVHIQTSVPTCHLLGDVQDPELEGGFAAISACDGLRGVFQLSNEDYFIEPLDEVPAQPGHAQPHMVYKHKRSGQQDDSRTSGTCGVQGSPELKHQREHWEQRQQKRRQQRSISKEKWVETLVVADSKMVEYHGQPQVESYVLTIMNMVAGLYHDPSIGNPIHITVVRLIILEDEEKDLKITHHADDTLKNFCRWQKNVNMKGDDHPQHHDTAILLTRKDLCATMNHPCETLGLSHVAGLCHPQLSCSVSEDTGLPLAFTVAHELGHSFGIQHDGTGNDCESIGKRPFIMSPQLLYDRGIPLTWSRCSREYITRFLDRGWGLCLDDRPSKGVINFPSVLPGVLYDVNHQCRLQYGPSSAYCEDVDNVCYTLWCSVGTTCHSKMDAAVDGTSCGKNKWCLNGECVPEGFQPETVDGGWSGWSAWSVCSRSCGVGVRSSERQCTQPVPKNKGKYCVGERKRYRLCNLQACPPDRPSFRHTQCSQFDSMLYKGKLHKWVPVLNDENPCELHCRPFNYSNREKLRDAVMDGTPCYQGRISRDICIDGICKKVGCDFELDSGAEEDRCGVCRGDGSTCHTVSRTFKEAEGMGYVDVGLIPAGAREILIEEVAEAANFLALRSEDPDKYFLNGGWTIQWNGDYQVAGTTFTYTRKGNWETLTSPGPTTEPVWIQLLFQERNPGVHYKYTIQRASHSEAQPPEFSWHYGPWSKCPVTCGTGVQRQSLYCMEKQAGIVDEGHCDHLSRPRDRKRKCNEEPCPARWWVGDWQPCSRSCGPGGFFRRAVFCTRSVGLDEQRALEPSACGHLPRPLAEIPCYHYVACPSSWGVGNWSQCSVTCGAGIRQRSVLCINNTGVPCDGAERPITETFCFLQPCQYSTYIVDTGASGSGSSSPELFNEVDFDPHQPVPRPSPASSPKPVSISNAIDEEDPELDPPGPVFVDDFYYDYNFINFHEDLSYGSFEESHSDLVDIGGQTVPPHIRPTEPPSDSPVPTAGAPGAEEEGIQGSWSPSPLLSEASHSPPVLLENTPVNPLANFLTEEESPIGAPELGLPSVSWPPASVDGMVTSVAPGNPDELLVREDTQSQPSTPWSDRNKLSKDGNPLGPTSPALPKSPFPTQPSSPSNSTTQASLSPDAVEVSTGWNVALDPVLEADLKPVHAPTDPGLLDQIQTPHTEGTQSPGLLPRPAQETQTNSSKDPAVQPLQPSLVEDGAPTDLLPAKNASWQVGNWSQCSTTCGLGAIWRLVRCSSGNDEDCTLSSRPQPARHCHLRPCAAWRAGNWSKCSRNCGGGSATRDVQCVDTRDLRPLRPFHCQPGPTKPPTRQLCGTQPCLPWYTSSWRECSEACGGGEQQRLVTCPEPGLCEESLRPNNTRPCNTHPCTQWVVGPWGQCSAPCGGGVQRRLVKCVNTQTGLAEEDSDLCSHEAWPESSRPCATEDCELVEPSRCERDRLPFNFCETLRLLGRCQLPTIRAQCCRSCPPLSRGVPSRGHQRVARR

SEQ ID NO: 23 - protein, 1657 aa, Artificial Sequence
  Mouse ADAMTS7 from Q68SA9
MHRGPSLLLILCALASRVLGPASGLVTEGRAGLDIVHPVRVDAGGSFLSYELWPRVLRKRDVSTTQASSAFYQLQYQGRELLFNLTTNPYLMAPGFVSEIRRHSTLGHAHIQTSVPTCHLLGDVQDPELEGGFAAISACDGLRGVFQLSNEDYFIEPLDGVSAQPGHAQPHVVYKHQGSRKQAQQGDSRPSGTCGMQVPPDLEQQREHWEQQQQKRRQQRSVSKEKWVETLVVADSKMVEYHGQPQVESYVLTIMNMVAGLFHDPSIGNPIHISIVRLIILEDEEKDLKITHHAEETLKNFCRWQKNINIKGDDHPQHHDTAILLTRKDLCASMNQPCETLGLSHVSGLCHPQLSCSVSEDTGMPLAFTVAHELGHSFGIQHDGTGNDCESIGKRPFIMSPQLLYDRGIPLTWSRCSREYITRFLDRGWGLCLDDRPSKDVIALPSVLPGVLYDVNHQCRLQYGSHSAYCEDMDDVCHTLWCSVGTTCHSKLDAAVDGTSCGKNKWCLKGECVPEGFQPEAVDGGWSGWSAWSDCSRSCGVGVRSSERQCTQPVPKNRGKYCVGERKRSQLCNLPACPPDRPSFRHTQCSQFDGMLYKGKLHKWVPVPNDDNPCELHCRPSNSSNTEKLRDAVVDGTPCYQSRISRDICLNGICKNVGCDFVIDSGAEEDRCGVCRGDGSTCQTVSRTFKETEGQGYVDIGLIPAGAREILIEEVAEAANFLALRSEDPDKYFLNGGWTIQWNGDYRVAGTTFTYARKGNWENLTSPGPTSEPVWIQLLFQEKNPGVHYQYTIQRDSHDQVRPPEFSWHYGPWSKCTVTCGTGVQRQSLYCMERQAGVVAEEYCNTLNRPDERQRKCSEEPCPPRWWAGEWQPCSRSCGPEGLSRRAVFCIRSMGLDEQRALELSACEHLPRPLAETPCNRHVICPSTWGVGNWSQCSVTCGAGIRQRSVLCINNTDVPCDEAERPITETFCFLQPCQYPMYIVDTGASGSGSSSPELFNEVDFIPNQLAPRPSPASSPKPVSISNAIDEEELDPPGPVFVDDFYYDYNFINFHEDLSYGSFEEPHPDLVDNGGWTAPPHIRPTESPSDTPVPTAGALGAEAEDIQGSWSPSPLLSEASYSPPGLEQTSINPLANFLTEEDTPMGAPELGFPSLPWPPASVDDMMTPVGPGNPDELLVKEDEQSPPSTPWSDRNKLSTDGNPLGHTSPALPQSPIPTQPSPPSISPTQASPSPDVVEVSTGWNAAWDPVLEADLKPGHGELPSTVEVASPPLLPMATVPGIWGRDSPLEPGTPTFSSPELSSQHLKTLTMPGTLLLTVPTDLRSPGPSGQPQTPNLEGTQSPGLLPTPARETQTNSSKDPEVQPLQPSLEEDGDPADPLPARNASWQVGNWSQCSTTCGLGAIWRLVSCSSGNDEDCTLASRPQPARHCHLRPCAAWRTGNWSKCSRNCGGGSSTRDVQCVDTRDLRPLRPFHCQPGPTKPPNRQLCGTQPCLPWYTSSWRECSEACGGGEQQRLVTCPEPGLCEESLRPNNSRPCNTHPCTQWVVGPWGQCSAPCGGGVQRRLVRCVNTQTGLAEEDSDLCSHEAWPESSRPCATEDCELVEPPRCERDRLSFNFCETLRLLGRCQLPTIRAQCCRSCPPLSRGVPSRGHQRVARR

SEQ ID NO: 24 - protein, 1594 aa, Artificial Sequence
  Human ADAMTS12 from P58397
MPCAQRSWLANLSVVAQLLNFGALCYGRQPQPGPVRFPDRRQEHFIKGLPEYHVVGPVRVDASGHFLSYGLHYPITSSRRKRDLDGSEDWVYYRISHEEKDLFFNLTVNQGFLSNSYIMEKRYGNLSHVKMMASSAPLCHLSGTVLQQGTRVGTAALSACHGLTGFFQLPHGDFFIEPVKKHPLVEGGYHPHIVYRRQKVPETKEPTCGLKDSVNISQKQELWREKWERHNLPSRSLSRRSISKERWVETLVVADTKMIEYHGSENVESYILTIMNMVTGLFHNPSIGNAIHIVVVRLILLEEEEQGLKIVHHAEKTLSSFCKWQKSINPKSDLNPVHHDVAVLLTRKDICAGFNRPCETLGLSHLSGMCQPHRSCNINEDSGLPLAFTIAHELGHSFGIQHDGKENDCEPVGRHPYIMSRQLQYDPTPLTWSKCSEEYITRFLDRGWGFCLDDIPKKKGLKSKVIAPGVIYDVHHQCQLQYGPNATFCQEVENVCQTLWCSVKGFCRSKLDAAADGTQCGEKKWCMAGKCITVGKKPESIPGGWGRWSPWSHCSRTCGAGVQSAERLCNNPEPKFGGKYCTGERKRYRLCNVHPCRSEAPTFRQMQCSEFDTVPYKNELYHWFPIFNPAHPCELYCRPIDGQFSEKMLDAVIDGTPCFEGGNSRNVCINGICKMVGCDYEIDSNATEDRCGVCLGDGSSCQTVRKMFKQKEGSGYVDIGLIPKGARDIRVMEIEGAGNFLAIRSEDPEKYYLNGGFIIQWNGNYKLAGTVFQYDRKGDLEKLMATGPTNESVWIQLLFQVTNPGIKYEYTIQKDGLDNDVEQQMYFWQYGHWTECSVTCGTGIRRQTAHCIKKGRGMVKATFCDPETQPNGRQKKCHEKACPPRWWAGEWEACSATCGPHGEKKRTVLCIQTMVSDEQALPPTDCQHLLKPKTLLSCNRDILCPSDWTVGNWSECSVSCGGGVRIRSVTCAKNHDEPCDVTRKPNSRALCGLQQCPSSRRVLKPNKGTISNGKNPPTLKPVPPPTSRPRMLTTPTGPESMSTSTPAISSPSPTTASKEGDLGGKQWQDSSTQPELSSRYLISTGSTSQPILTSQSLSIQPSEENVSSSDTGPTSEGGLVATTTSGSGLSSSRNPITWPVTPFYNTLTKGPEMEIHSGSGEEREQPEDKDESNPVIWTKIRVPGNDAPVESTEMPLAPPLTPDLSRESWWPPFSTVMEGLLPSQRPTTSETGTPRVEGMVTEKPANTLLPLGGDHQPEPSGKTANRNHLKLPNNMNQTKSSEPVLTEEDATSLITEGFLLNASNYKQLTNGHGSAHWIVGNWSECSTTCGLGAYWRRVECSTQMDSDCAAIQRPDPAKRCHLRPCAGWKVGNWSKCSRNCSGGFKIREIQCVDSRDHRNLRPFHCQFLAGIPPPLSMSCNPEPCEAWQVEPWSQCSRSCGGGVQERGVFCPGGLCDWTKRPTSTMSCNEHLCCHWATGNWDLCSTSCGGGFQKRTVQCVPSEGNKTEDQDQCLCDHKPRPPEFKKCNQQACKKSADLLCTKDKLSASFCQTLKAMKKCSVPTVRAECCFSCPQTHITHTQRQRRQRLLQKSKEL

SEQ ID NO: 25 - protein, 1599 aa, Artificial Sequence
  Rat ADAMTS12 from D3ZTJ3
MPCAQGNWMAKLSMVAQLLNFGAFCHGRQAQPWPVRFPDPKQEHFIKSLPEYHIVSPVQVDASGHFLSYGLHHPVTGSRKKRAAGGSGDQVYYRISHEEKNLFFNLTVNWEFLSNGYVVERRYGNLSHVKMAASSGQPCHLRGTVLQQGPTIRMGTAALSACQGLTGFFHLPHGDFFIEPVKKHPLTEEGYQPHVIYRRQSYRVPETKEPTCGLKDSLDNSVKQELQREKWERKNWPSRSLSRRSISKERWVETLVVADTKMVEYHGSENVESYILTIMNMVTGLFHNPSIGNAVHIVVVRLILLEEEEQGLKIVHHAEKTLSSFCKWQKSINPKSDLNPVHHDVAVLITRKDICAGVNRPCETLGLSQLSGMCQPHRSCNINEDSGLPLAFTIAHELGHSFGIQHDGKENDCEPVGRHPYIMSQQIQYDPTPLTWSKCSKEYITRFLDRGRGFCLDDVPRKKGLKSNVIAPGVIYDVHHQCQLQYGPNATFCQEVENVCQTLWCSVKGFCRSKLDAAADGTRCGEKKWCMAGKCITVGKKPESIPGGWGRWSPWSHCSRTCGAGAQSAERLCNNPEPKFGGKYCTGERKRYRLCNVHPCRSDTPTFRQMQCSEFDTVPYKNQFYRWFPVFNPAHPCELYCRPIDEQFSERMLEAVIDGTPCFEGGNSRNVCINGICKRVGCDYEIDSNATEDRCGVCLGDGSACQTVKKVFRQKEGSGYIDIGLIPKGARDIRVMEIKAAGNFLAIRSEDPEKYYLNGGFIIQWNGNYKLAGTVFQYDRKGDLERLMAPGPTNESVWLQLLFQVTNPGIKYEYTVRKDGLDNDVEKLLYFWQFGRWTECSVTCGTGIRRQTAHCVKKGHGIVKTTFCNPETQPSVRQKKCYEKDCPPRWWAGEWEACSMTCGPYGEKKRTVLCIQTMGSDEQALPATDCQHLLKPKTLVSCNRDILCPSDWTVGNWSECSVSCGGGVRIRSVTCAKNLNEPCDKTRKPNSRALCGLQQCPFSRRVLKPNKDTVPSGKNPTTSEHDHFKPIPASTSRPTPLSTPTVPESVSTSTPTINSLGSTITSQEEPDGIGWQNNSTQAEEDSHIPTSVGSTSQTPLTSWSWSMQPDDENVSSSAIGPTSESDFWATTSDSGLSSSNAMTWQVTPFYSTATTEPEVEIHSGSGEDSDQPLNKEENNSVLWNKIRVPERDAPMEMDAEIPLGPPPTSYVTEESSWPPFSTMMKSSLPAWSFKNETPRDEGMITEKSGNIPLPLGGDHQTTSPEKLGNNDQLASANSTNPTQGSGPVLTEEDASTLIEEGFLLNASNYKHLMKDHSPAHWIVGNWSKCSTTCGLGAYWRSVECSTGMNADCAAIQRPDPAKKCHLRPCAGWRVGNWSKCSRNCSGGFKIREVQCMDGVDHHRSLRPFHCQFLAGVPPPLSMSCNLEPCEEWKVEPWSQCSRSCGGGVQERGVFCPGGLCDWTKRPASTVPCNRHLCCHWATGNWELCTTSCGGGSQKRTVHCIPSENSTTEDQDQCFCDHQARPPEFQNCNQQACRKSADLTCTKDRLSTSFCQTLKSMKKCSVPSVRVQCCLSCPQTQSIHTQRQRKQQMLQNHDTL

SEQ ID NO: 26 - protein, 1600 aa, Artificial Sequence
  Mouse ADAMTS12 from Q811B3
MPCARGSWLAKLSIVAQLINFGAFCHGRQTQPWPVRFPDPRQEHFIKSLPEYHIVSPVQVDAGGHVLSYGLHHPVTSSRKKRAAGGSGDQLYYRISHEEKDLFFNLTVNWEFLSNGYVVEKRYGNLSHVKMVASSGQPCHLRGTVLQQGTTVGIGTAALSACQGLTGFFHLPHGDFFIEPVKKHPLTEEGSYPHVVYRRQSIRAPETKEPICGLKDSLDNSVKQELQREKWERKTLRSRSLSRRSISKERWVETLVVADTKTVEYHGSENVESYILTIMNMVTGLFHSPSIGNLVHIVVVRLILLEEEEQGLKIVHHAEKTLSSFCKWQKSINPKSDLNPVHHDVAVLITRKDICAGVNRPCETLGLSQLSGMCQPHRSCNINEDSGLPLAFTIAHELGHSFGIQHDGKENDCEPVGRHPYIMSQQIQYDPTPLTWSKCSKEYITRFLDRGRGFCLDDIPSKKGLKSNVIAPGVIYDVHHQCQLQYGPNATFCQEVENVCQTLWCSVKGFCRSKLDAAADGTRCGEKKWCMAGKCITVGKKPESIPGGWGRWSPWSHCSRTCGAGAQSAERLCNNPEPKFGGKYCTGERKRYRLCNVHPCRSDTPTFRQMQCSEFDTVPYKNQFYRWFPVFNAAHPCELYCRPIDEQFSERMLEAVIDGTPCFEGGNSRNVCINGICKRVGCDYEIDSNATEDRCGVCLGDGSACQTVKKLFRQKEGSGYVDIGLIPKGARDIRVMEIKAAGNFLAIRSEDPEKYYLNGGFIIQWNGNYKLAGTVFQYDRKGDLEKLIAPGPTNESVWLQLLFQVTNPGIKYEYTVRKDGLDNDVEKLLYFWQFGRWTECSVTCGTGIRRQAAHCVKKGHGIVKTTFCNPETQPSVRQKKCHEKDCPPRWWAGEWEACSTTCGPYGEKKRTVLCIQTMGSDEQALPATDCQHLLKPKALVSCNRDILCPSDWTVGNWSECSVSCGGGVRIRSVTCAKNLNEPCDKTRKPNSRALCGLQQCPFSRRVLKPNKDIAPSGKNQSTAEHDPFKPIPAPTSRPTPLSTPTVPESMSTSTPTINSLGSTIASQEDANGMGWQNNSTQAEEGSHFPTSSGSTSQVPVTSWSLSIQPDDENVSSSAIGPTSEGDFWATTTSDSGLSSSDAMTWQVTPFYSTMTTDPEVEIHSGSGEDSDQPLNKDKSNSVIWNKIGVPEHDAPMETDAELPLGPPPTSYMGEEPSWPPFSTKMEGSLPAWSFKNETPRDDGMIAEKSRKIPLPLAGDHHPATSEKLENHDKLALPNTTNPTQGFGPVLTEEDASNLIAEGFLLNASDYKHLMKDHSPAYWIVGNWSKCSTTCGLGAYWRSVECSSGVDADCTTIQRPDPAKKCHLRPCAGWRVGNWSKCSRNCSGGFKIREVQCMDSLDHHRSLRPFHCQFLAGAPPPLSMSCNLEPCGEWQVEPWSQCSRSCGGGVQERGVSCPGGLCDWTKRPATTVPCNRHLCCHWATGNWELCNTSCGGGSQKRTIHCIPSENSTTEDQDQCLCDHQVKPPEFQTCNQQACRKSADLTCLKDRLSISFCQTLKSMRKCSVPSVRAQCCLSCPQAPSIHTQRQRKQQLLQNHDML

SEQ ID NO: 27 - protein, 202 aa, Artificial Sequence
  Human ADAMTS7 Pro Domain (hADAMTS7_Pro)
RATEGRAALDIVHPVRVDAGGSFLSYELWPRALRKRDVSVRRDAPAFYELQYRGRELRFNLTANQHLLAPGFVSETRRRGGLGRAHIRAHTPACHLLGEVQDPELEGGLAAISACDGLKGVFQLSNEDYFIEPLDSAPARPGHAQPHVVYKRQAPERLAQRGDSSAPSTCGVQVYPELESRRERWEQRQQWRRPRLRRLHQR

SEQ ID NO: 28 - protein, 193 aa, Artificial Sequence
  Rat ADAMTS7 Pro Domain (rADAMTS7_Pro)
LPTEGRAGLDIVHPVRVDAGGSFLSYELWPRVLRKRDVSAAQASSAFYQLQYQGRELLFNLTTNPYLLAPGFVSEIRRRSNLSNVHIQTSVPTCHLLGDVQDPELEGGFAAISACDGLRGVFQLSNEDYFIEPLDEVPAQPGHAQPHMVYKHKRSGQQDDSRTSGTCGVQGSPELKHQREHWEQRQQKRRQQR

SEQ ID NO: 29 - protein, 301 aa, Artificial Sequence
  Human ADAMTS7 CD domain (hADAMTS7_CD)
SVSKEKWVETLVVADAKMVEYHGQPQVESYVLTIMNMVAGLFHDPSIGNPIHITIVRLVLLEDEEEDLKITHHADNTLKSFCKWQKSINMKGDAHPLHHDTAILLTRKDLCAAMNRPCETLGLSHVAGMCQPHRSCSINEDTGLPLAFTVAHELGHSFGIQHDGSGNDCEPVGKRPFIMSPQLLYDAAPLTWSRCSRQYITRFLDRGWGLCLDDPPAKDIIDFPSVPPGVLYDVSHQCRLQYGAYSAFCEDMDNVCHTLWCSVGTTCHSKLDAAVDGTRCGENKWCLSGECVPVGFRPEAV

SEQ ID NO: 30 - protein, 302 aa, Artificial Sequence
  Rat ADAMTS7 CD domain (rADAMTS7_CD)
SISKEKWVETLVVADSKMVEYHGQPQVESYVLTIMNMVAGLYHDPSIGNPIHITVVRLIILEDEEKDLKITHHADDTLKNFCRWQKNVNMKGDDHPQHHDTAILLTRKDLCATMNHPCETLGLSHVAGLCHPQLSCSVSEDTGLPLAFTVAHELGHSFGIQHDGTGNDCESIGKRPFIMSPQLLYDRGIPLTWSRCSREYITRFLDRGWGLCLDDRPSKGVINFPSVLPGVLYDVNHQCRLQYGPSSAYCEDVDNVCYTLWCSVGTTCHSKMDAAVDGTSCGKNKWCLNGECVPEGFQPETV

SEQ ID NO: 31 - protein, 562 aa, Artificial Sequence
  rPro-hCD (Rat 1-217/Human 237-537 (R58A/R60A/R217A))-TEV-2Strep-6His
MHRGLNLLLILCALAPHVLGPASGLPTEGRAGLDIVHPVRVDAGGSFLSYELWPRVLAKADVSAAQASSAFYQLQYQGRELLFNLTTNPYLLAPGFVSEIRRRSNLSNVHIQTSVPTCHLLGDVQDPELEGGFAAISACDGLRGVFQLSNEDYFIEPLDEVPAQPGHAQPHMVYKHKRSGQQDDSRTSGTCGVQGSPELKHQREHWEQRQQKRRQQASVSKEKWVETLVVADAKMVEYHGQPQVESYVLTIMNMVAGLFHDPSIGNPIHITIVRLVLLEDEEEDLKITHHADNTLKSFCKWQKSINMKGDAHPLHHDTAILLTRKDLCAAMNRPCETLGLSHVAGMCQPHRSCSINEDTGLPLAFTVAHELGHSFGIQHDGSGNDCEPVGKRPFIMSPQLLYDAAPLTWSRCSRQYITRFLDRGWGLCLDDPPAKDIIDFPSVPPGVLYDVSHQCRLQYGAYSAFCEDMDNVCHTLWCSVGTTCHSKLDAAVDGTRCGENKWCLSGECVPVGFRPEAVGSENLYFQSGWSHPQFEKGGGSGGGSGGGSWSHPQFEKHHHHHH

SEQ ID NO: 32 - protein, 196 aa, Artificial Sequence
  Mouse ADAMTS-7 prodomain (Mouse_Pro)
LVTEGRAGLDIVHPVRVDAGGSFLSYELWPRVLRKRDVSTTQASSAFYQLQYQGRELLFNLTTNPYLMAPGFVSEIRRHSTLGHAHIQTSVPTCHLLGDVQDPELEGGFAAISACDGLRGVFQLSNEDYFIEPLDGVSAQPGHAQPHVVYKHQGSRKQAQQGDSRPSGTCGMQVPPDLEQQREHWEQQQQKRRQQR

SEQ ID NO: 33 - protein, 45 aa, Artificial Sequence
  TSP-1 candidate region
CDELSSMVLELRGLRTIVTTLQDSIRKVTEENKELANELRRPPLC